European Patent Specification EP 3 336 096 B1, published September 23, 2026. Title: COMPOSITIONS COMPRISING IMPROVED IL-12 GENETIC CONSTRUCTS AND VACCINES, IMMUNOTHERAPEUTICS AND METHODS OF USING THE SAME. Applicant: The Turstees of the University of Pennsylvania. The sequence listing filed with the application follows.

SEQUENCE LISTING (5 sequences)

SEQ ID NO: 1 - DNA, 660 bp, Artificial Sequence
  IL-12 Optimized p35 subunit nucleic acid
atgtgccccgctcggtccctgctgctggtcgctaccctggtcctgctggatcacctgtcactggctcgaaatctgcctgtcgctacccccgatcctggcatgttcccctgcctgcaccatagccagaacctgctgcgggccgtgtccaatatgctgcagaaagctagacagacactggagttttacccttgtacttctgaggaaatcgaccacgaggatattactaaggacaaaacctccacagtcgaagcctgcctgccactggagctgaccaagaacgaatcatgtctgaatagcagggagacttccttcatcaccaacgggtcttgcctggctagtcgcaagaccagcttcatgatggcactgtgcctgagctccatctacgaggatctgaagatgtatcaggtggaattcaaaaccatgaacgctaagctgctgatggaccctaaacgacagatctttctggatcagaatatgctggcagtgattgacgagctgatgcaggccctgaacttcaatagcgaaaccgtcccacagaagtctagtctggaggaacccgacttttataagacaaaaatcaagctgtgcattctgctgcatgcctttcggattcgggctgtcactattgatcgggtcatgtcatacctgaacgcttcctaa

SEQ ID NO: 2 - protein, 219 aa, Artificial Sequence
  IL-12 Opt p35 subunit amino acid
MCPARSLLLVATLVLLDHLSLARNLPVATPDPGMFPCLHHSQNLLRAVSNMLQKARQTLEFYPCTSEEIDHEDITKDKTSTVEACLPLELTKNESCLNSRETSFITNGSCLASRKTSFMMALCLSSIYEDLKMYQVEFKTMNAKLLMDPKRQIFLDQNMLAVIDELMQALNFNSETVPQKSSLEEPDFYKTKIKLCILLHAFRIRAVTIDRVMSYLNAS

SEQ ID NO: 3 - DNA, 987 bp, Artificial Sequence
  IL-12 Opt p40 subunit nucleic acid
atgtgccatcagcagctggtcatctcttggtttagtctggtgtttctggcttctccactggtcgctatctgggaactgaaaaaggatgtgtacgtggtcgagctggactggtatccagatgcacccggagaaatggtggtcctgacctgcgacacacccgaggaagatggcatcacttggaccctggaccagagctccgaggtgctgggatctggcaagacactgactattcaggtcaaagaattcggggatgccggacagtacacatgtcacaagggcggggaggtgctgagtcactcactgctgctgctgcataagaaagaagacggcatctggtctactgacattctgaaggatcagaaagagcctaagaacaaaaccttcctgagatgcgaagctaagaattatagtgggaggtttacctgttggtggctgaccacaatctcaactgacctgacctttagcgtgaaatctagtagggggtcaagcgatccacagggagtgacctgcggagcagctacactgagcgccgagcgggtgagaggagacaacaaggagtacgaatatagtgtcgagtgccaggaagattcagcctgtcccgcagccgaggaatccctgcctatcgaagtgatggtggacgctgtgcacaagctgaaatacgaaaactacacatcctctttctttattcgcgacatcattaagccagatccccctaaaaacctgcagctgaagcccctgaaaaattcccgacaggtggaggtctcttgggaataccctgatacatggagcactccacattcttatttcagtctgactttttgcgtgcaggtccagggcaagagcaaaagggagaagaaagaccgcgtgttcaccgataagacatccgctactgtcatctgtcgaaaaaacgcaagcatttccgtgcgggcacaggataggtattattccagcagttggtctgagtgggcttccgtcccttgtagttga

SEQ ID NO: 4 - protein, 328 aa, Artificial Sequence
  IL-12 Opt p40 subunit amino acid
MCHQQLVISWFSLVFLASPLVAIWELKKDVYVVELDWYPDAPGEMVVLTCDTPEEDGITWTLDQSSEVLGSGKTLTIQVKEFGDAGQYTCHKGGEVLSHSLLLLHKKEDGIWSTDILKDQKEPKNKTFLRCEAKNYSGRFTCWWLTTISTDLTFSVKSSRGSSDPQGVTCGAATLSAERVRGDNKEYEYSVECQEDSACPAAEESLPIEVMVDAVHKLKYENYTSSFFIRDIIKPDPPKNLQLKPLKNSRQVEVSWEYPDTWSTPHSYFSLTFCVQVQGKSKREKKDRVFTDKTSATVICRKNASISVRAQDRYYSSSWSEWASVPCS

SEQ ID NO: 5 - protein, 18 aa, Artificial Sequence
  IgE leader
MDWTWILFLVAAATRVHS